European Patent Specification EP 3 730 513 B1, published June 5, 2024. Title: Péptido y composiciones farmacéuticas del mismo para uso como antimicrobiano y en el tratamiento del cáncer. Applicant: Universitat de València. The sequence listing filed with the application follows.

SEQUENCE LISTING (2 sequences)

SEQ ID NO: 1 - protein, 31 aa, Secuencia Artificial
  Tribolium castaneum Defensina 3; fragmento PaSK
KVNHAACAAHCLLKRKRGGYCNKRRICVCRN

SEQ ID NO: 2 - protein, 29 aa, Secuencia Artificial
  Tribolium castaneum Defensina 3; fragmento TcDef3-pep
VNHAACAAHCLLKRKRGGYCNKRRICVCR